European Patent Specification EP 3 902 915 B1, published August 23, 2023. Title: Method for selecting cells based on CRISPR/Cas-mediated integration of a detectable tag to a target protein. Applicant: F. Hoffmann-La Roche AG Hoffmann-La Roche Inc. The sequence listing filed with the application follows.

SEQUENCE LISTING (35 sequences)

SEQ ID NO: 1 - DNA, 26 bp, Artificial Sequence
  gRNA1 forward
gatcggagtgcatctccatccacgtg

SEQ ID NO: 2 - DNA, 26 bp, Artificial Sequence
  gRNA1 reverse
aaaacacgtggatggagatgcactcc

SEQ ID NO: 3 - DNA, 26 bp, Artificial Sequence
  gRNA2 forward
gatcgggccaggctggtgtccagatg

SEQ ID NO: 4 - DNA, 26 bp, Artificial Sequence
  gRNA2 reverse
aaaacatctggacaccagcctggccc

SEQ ID NO: 5 - DNA, 26 bp, Artificial Sequence
  gRNA3 forward
gatcggagctctactgcctggaacag

SEQ ID NO: 6 - DNA, 26 bp, Artificial Sequence
  gRNA3 reverse
aaaactgttccaggcagtagagctcc

SEQ ID NO: 7 - DNA, 20 bp, Artificial Sequence
  crRNA1
gagtgcatctccatccacgt

SEQ ID NO: 8 - DNA, 20 bp, Artificial Sequence
  crRNA2
ggccaggctggtgtccagat

SEQ ID NO: 9 - DNA, 20 bp, Artificial Sequence
  crRNA3
gagctctactgcctggaaca

SEQ ID NO: 10 - DNA, 55 bp, Artificial Sequence
  D_Hygro fwd
cgaatgcggccgcagaagcaataagaggactgcggaagagctccctgtcaatgta

SEQ ID NO: 11 - DNA, 50 bp, Artificial Sequence
  D_Hygro rev
gccttaattaaagtgctccagggtggtgtgggtggtgaggatggagttgt

SEQ ID NO: 12 - DNA, 40 bp, Artificial Sequence
  D_5´HA fwd
gacattgattattgaaagcaataagaggactgcggaagag

SEQ ID NO: 13 - DNA, 40 bp, Artificial Sequence
  D_5´HA rev
tgctcacctgcgggaaggaaaaaagatatcacaatttaaa

SEQ ID NO: 14 - DNA, 40 bp, Artificial Sequence
  D_eGFP fwd
tcccgcaggtgagcaagggcgaggaactgttcaccggggt

SEQ ID NO: 15 - DNA, 45 bp, Artificial Sequence
  D_eGFP_rev
actcacggctgcctcccccgcctttgtacagttcgtccattccga

SEQ ID NO: 16 - DNA, 80 bp, Artificial Sequence
  D_3´HA fwd
aaaggcgggggaggcagccgtgaatgtataagtatacatgtgggacaagcaggagtacaaatcggcaatgcctgctggga

SEQ ID NO: 17 - DNA, 40 bp, Artificial Sequence
  D_3´HA rev
cttttgctcacggccagtgctccagggtggtgtgggtggt

SEQ ID NO: 18 - DNA, 49 bp, Artificial Sequence
  D_3´HA-Z fwd
gtcatcaatagattggtttaaattgtgatatcttttttccttcccgcag

SEQ ID NO: 19 - DNA, 50 bp, Artificial Sequence
  D_3'HA-Z rev
aaccagaaagctttaacgtctgtcagttaagctgaagctgaaattctggg

SEQ ID NO: 20 - DNA, 40 bp, Artificial Sequence
  QuickChange fwd
tgcctgctgggaattatattgtttagagcatggcatccag

SEQ ID NO: 21 - DNA, 40 bp, Artificial Sequence
  QuickChange rev
ctggatgccatgctctaaacaatataattcccagcaggca

SEQ ID NO: 22 - DNA, 34 bp, Artificial Sequence
  eGFP fwd
ggccgacaagcagaaaaacggcatcaaagtgaac

SEQ ID NO: 23 - DNA, 26 bp, Artificial Sequence
  TUBA1B Exon4 rev
ggcggttaaggttagtgtaggttggg

SEQ ID NO: 24 - DNA, 34 bp, Artificial Sequence
  cDNA fwd
atggtgagcaagggcgaggaactgttcaccgggg

SEQ ID NO: 25 - DNA, 28 bp, Artificial Sequence
  cDNA rev
ttagtattcctctccttcttcctcaccc

SEQ ID NO: 26 - DNA, 20 bp, Artificial Sequence
  Hygro fwd
accgcaaggaatcggtcaat

SEQ ID NO: 27 - DNA, 20 bp, Artificial Sequence
  Hygro rev
tgctgctccatacaagccaa

SEQ ID NO: 28 - DNA, 33 bp, Artificial Sequence
  Cas9 fwd
ccctgctgttcgacagcggcgaaacagccgagg

SEQ ID NO: 29 - DNA, 39 bp, Artificial Sequence
  Cas9 rev
ggcatcctcggccaggtcgaagttgctcttgaagttggg

SEQ ID NO: 30 - DNA, 33 bp, Artificial Sequence
  eGFP_2 fwd
gacctacggcgtgcagtgcttcagcagataccc

SEQ ID NO: 31 - DNA, 34 bp, Artificial Sequence
  eGFP_2 rev
gttcactttgatgccgtttttctgcttgtcggcc

SEQ ID NO: 32 - protein, 239 aa, Artificial Sequence
  eGFP-Tag
MVSKGEELFTGVVPILVELDGDVNGHKFSVSGEGEGDATYGKLTLKFICTTGKLPVPWPTLVTTLTYGVQCFSRYPDHMKQHDFFKSAMPEGYVQERTIFFKDDGNYKTRAEVKFEGDTLVNRIELKGIDFKEDGNILGHKLEYNYNSHNVYIMADKQKNGIKVNFKIRHNIEDGSVQLADHYQQNTPIGDGPVLLPDNHYLSYQSALSKDPNEKRDHMVLLEFVTAAGITLGMDELYK

SEQ ID NO: 33 - DNA, 717 bp, Artificial Sequence
  eGFP-tag nuc
atggtgagcaagggcgaggaactgttcaccggggtcgtgcccatcctcgttgagctggacggagatgtgaacggccacaaattttccgtctctggggaaggtgagggcgacgccacatacggaaagcttactctgaaattcatttgcaccacagggaagttgcctgtgccatggcccactctcgtaaccacactgacgtatggcgtgcagtgttttagtagataccctgatcatatgaaacagcacgactttttcaagagtgccatgccagaaggttatgtgcaggagcggacgatctttttcaaggatgacggcaattacaaaaccagagcagaggtcaagtttgaaggggatacacttgtgaaccgcattgagctgaaaggaatcgacttcaaggaagatggcaatatactcgggcataaactggagtataactacaatagccacaacgtttacatcatggccgacaagcagaagaatggtattaaagtgaacttcaagatcaggcacaatattgaggacggctccgtccaattggctgatcattatcagcagaacactcccatcggagacgggcctgtgctgctcccagataatcactacctgtcttatcagtcagcacttagcaaagacccgaacgaaaagcgggatcatatggttctgttggagtttgtaaccgcggctggcataacactcggaatggacgaactgtacaaa

SEQ ID NO: 34 - RNA, 22 nt, Artificial Sequence
  Cas9
guuuuagagcurugyuguuuug

SEQ ID NO: 35 - DNA, 83 bp, Artificial Sequence
  eGFP exaon 2 start
ctgagtgcatctccatccacgttggccaggctggtgtccagattggcaatgcctgctgggagctctactgcctggaacacggc